European Patent Specification EP 4 127 157 B1, published February 11, 2026. Title: MODIFIED DIPEPTIDE CLEAVASES, USES THEREOF AND RELATED KITS. Applicant: Encodia, Inc. The sequence listing filed with the application follows.

SEQUENCE LISTING (55 sequences)

SEQ ID NO: 1 - protein, 6 aa, Artificial Sequence
  DPP3 motif
  MISC_FEATURE (3)..(4): Xaa can be any naturally occurring amino acid
HEXXGH

SEQ ID NO: 2 - protein, 6 aa, Artificial Sequence
  DPP3 motif
  MISC_FEATURE (3)..(3): Xaa can be any naturally occurring amino acid
  MISC_FEATURE (6)..(6): Xaa can be naturally occurring glutamic acid (Glu) or aspartic acid (Asp)
EEXRAX

SEQ ID NO: 3 - DNA, 20 bp, Artificial Sequence
  P5 primer
aatgatacggcgaccaccga

SEQ ID NO: 4 - DNA, 24 bp, Artificial Sequence
  P7 primer
caagcagaagacggcatacgagat

SEQ ID NO: 5 - protein, 737 aa, Homo sapiens
  Dipeptidyl peptidase 3 (DPP3) (1)..(737): UniProt Accession No. Q9NY33
MADTQYILPNDIGVSSLDCREAFRLLSPTERLYAYHLSRAAWYGGLAVLLQTSPEAPYIYALLSRLFRAQDPDQLRQHALAEGLTEEEYQAFLVYAAGVYSNMGNYKSFGDTKFVPNLPKEKLERVILGSEAAQQHPEEVRGLWQTCGELMFSLEPRLRHLGLGKEGITTYFSGNCTMEDAKLAQDFLDSQNLSAYNTRLFKEVDGEGKPYYEVRLASVLGSEPSLDSEVTSKLKSYEFRGSPFQVTRGDYAPILQKVVEQLEKAKAYAANSHQGQMLAQYIESFTQGSIEAHKRGSRFWIQDKGPIVESYIGFIESYRDPFGSRGEFEGFVAVVNKAMSAKFERLVASAEQLLKELPWPPTFEKDKFLTPDFTSLDVLTFAGSGIPAGINIPNYDDLRQTEGFKNVSLGNVLAVAYATQREKLTFLEEDDKDLYILWKGPSFDVQVGLHELLGHGSGKLFVQDEKGAFNFDQETVINPETGEQIQSWYRSGETWDSKFSTIASSYEECRAESVGLYLCLHPQVLEIFGFEGADAEDVIYVNWLNMVRAGLLALEFYTPEAFNWRQAHMQARFVILRVLLEAGEGLVTITPTTGSDGRPDARVRLDRSKIRSVGKPALERFLRRLQVLKSTGDVAGGRALYEGYATVTDAPPECFLTLRDTVLLRKESRKLIVQPNTRLEGSDVQLLEYEASAAGLIRSFSERFPEDGPELEEILTQLATADARFWKGPSEAPSGQA

SEQ ID NO: 6 - protein, 710 aa, Saccharomyces cerevisiae
  Dipeptidyl peptidase 3 (DPP3) (1)..(710): UniProt Accession No. Q08225
MSHFFADHDAPLSMLSVKTEYFPQLTDKEQKYAHFMSKASHAGSRVVMRQVSHESEPIFDLILAIHSKLNGKYPEDDITQKQQTGLYLEYVSQFLSNLGNFKSFGDTKFIPRCEVKFFKQLLELAKINPCSSPLTLSPVDVNHEFTSHHLFSTINELIDIGIYHVEEKAALLGFPSQGYTSAYYLGLPVTPEDMALLKEQLFAELAILPENTRINKVGENSFQIWVASENVKNQITETYPSGQITLSNAVTKVEFIFGDHSREMRLVASYLKEAQKFAANDTQKAMLQEYINHFVTGSSQAHKEAQKLWVKDISPVIETNIGFIETYREPSGIIGEFESLVAIQNKERTAKFSSVNNAEEFISLLPWSKDYEKPIFNPPDFTSLEVLTFTGSGIPAGINIPNYDDVRLKIGFKNVSLGNILSAAAKSSSKHPPSFISQEDRPIFEKYQSDSFEVQVGIHELLGHGSGKLLTEFTDGFNFDKENPPLGLDGKPVSTYYKVGETWGSKFGQLAGPFEECRAEVIAMFLLTNKKILDIFGFHDVESQDKVIYAGYLQMARAGLLALEYWNPKTGKWGQPHMQARFSIMKTFMKHSTDKNFLKLEMNSTNDDFAIKLDKSLIKTAGHECVKDYLKHLHVYKCSGDVEQGSKYFIDRSTVTPDLASLRDIVLSKRLPRRQFIQSNSYIDDNNKVTLKEYDETPQGMLQSFLDREL

SEQ ID NO: 7 - protein, 674 aa, Bacteroides thetaiotaomicron
  Dipeptidyl peptidase 3 (DPP3) (1)..(674): UniProt Accession No. Q8A6N1
MAVTATILASCGGAKTTTAEADKFDYTVEQFADLQILRYKVPEFETLTLKQKELVYYLTQAALEGRDILFDQNGKYNLRIRRMLEAVYTNYKGDKSAPDFKNMEVYLKRVWFSNGIHHHYGMEKFVPGFSQDFLKQAVLGTDAQLLPLSEGQTAEQLCDELFPVMFDPAILAKRVNQADGEDLVLTSACNYYDGVTQQEAESFYGAMKDPKDETPVSYGLNSRLVKEDGKQEKVWKVGGLYTQAIEKIVYWLKKAETVAENDAQKAVISKLIQFYETGSLKDFDEYAILWVKDLDSRIDFVNGFTESYGDPLGVKASWESLVNFKDLDATHRTEIISSNAQWFEDHSPVDKSFKKEKVKGVSAKVITAAILAGDLYPATAIGINLPNANWIRAHHGSKSVTIGNITDAYNKAAHGNGFNEEFVCNDEERQRIDQYGDLTGELHTDLHECLGHGSGKLLPGVDPDALKAYGSTIEEARADLFGLYYVADPKLVELKLVPDAEAYKAEYYTFLMNGLMTQLVRIEPGNNIEEAHMRNRQLIARWVFEKGAPDKVVEMVKKDGKTYVVVNDYEKVRQLFGELLAEIQRIKSTGDFEGARTLVENYAVKVDPALHAEVLARYKKLNLAPYKGFINPVYELVTDKDGNITDVTVSYNEDYVEQMLRYSKDYSPLPSVNN

SEQ ID NO: 8 - protein, 558 aa, Caldithrix abyssi
  Dipeptidyl peptidase 3 (DPP3) (1)..(558): UniProt Accession No. H1XW48
MKRILLVLLTLVFLGAIACQKKEENKTEMVKLKRMIAQFAPTEIKYDHSLLDERKQKVVENLYRAAKIMDEIFLDQVYSKNFEIREQLRASSDPLDQLRLEYFTIMFGPFDRLNHDKPFIGNTPKPKGANFYPPDMTREEFENWLKAHPEDEAAFTSEFTVIRRQDGKLVAIPYSEYYKEYLTRAADYLKKAAEFADNPSLKKYLQLRAEAFLNNDYYESDLAWMDLNDHTIEVVIGPYEVYEDKLFNYKAAFEAFITLRDPVESAKLKKFVGYLDEMEKNLPIPDAYKNFNRGSESPMVVVQEVFSAGDTKAGVQTLAFNLPNDERVREAKGSKKVMLKNIHEAKFDKLLKPIAEKVLFAEQLPLVTFEGFFNHTLMHEISHGLGPGKIVLNGRQTEVKKELKETYSSIEECKADVLGMYNNLFMIEKGVYPPEFEKQIYVTFLAGIFRTIRFGINEAHGAGNAVIFNYLLEKGAYQFDPAAHRVKVNFEKIKDGVRDLANKVLTIQAQGDYMAAKNLLETYAVESEPIMIMRARLQELPVDIKPIFQIEKELGNSN

SEQ ID NO: 9 - protein, 8 aa, Artificial Sequence
  Substrate Sequence
DRVYIHPF

SEQ ID NO: 10 - protein, 703 aa, Aspergillus fumigatus
  Dipeptidyl peptidase 5 (DPP5) (1)..(703): Uniprot accession P0C959
LTPEQLITAPRRSEAIPDPSGKVAVFSTSQYSFETHKRTSWWSLLDLKTGQTKVLTNDSSVSEIVWLSDDSILYVNSTNADIPGGVELWVTQASSFAKGYKAASLPASFSGLKTAKTKSGDIRFVAYGQSYPNGTAYNEELATAPLSSARIYDSIYVRHWDYWLSTTFNAVFSGTLKKGHGKNGYSLDGELKNLVSPVKNAESPYPPFGGASDYDLSPDGKWVAFKSKAPELPKANFTTSYIYLVPHDASETARPINGPDSPGTPKGIKGDSSSPVFSPNGDKLAYFQMRDETYESDRRVLYVYSLGSKKTIPSVAGDWDRSPDSVKWTPDGKTLIVGSEDLGRTRLFSLPANAKDDYKPKNFTDGGSASAYYFLPDSSLLVTGSALWTNWNVYTAKPEKGVIKKIASANEIDPELKGLGPSDISEFYFQGNFTDIHAWVIYPENFDKSKKYPLIFFIHGGPQGNWADGWSTRWNPKAWADQGYVVVAPNPTGSTGFGQALTDAIQNNWGGAPYDDLVKCWEYVHENLDYVDTDHGVAAGASYGGFMINWIQGSPLGRKFKALVSHDGTFVADAKVSTEELWFMQREFNGTFWDARDNYRRWDPSAPERILQFATPMLVIHSDKDYRLPVAEGLSLFNVLQERGVPSRFLNFPDENHWVVNPENSLVWHQQALGWINKYSGVEKSNPNAVSLEDTVVPVVNYN

SEQ ID NO: 11 - protein, 689 aa, Porphyromonas gingivalis
  Dipeptidyl peptidase 7 (DPP7) (1)..(689): UniProt Accession No. B2RKV3
ADKGMWLLNELNQENLDRMRELGFTLPLDSLYSFDKPSIANAVVIFGGGCTGITVSDQGLIFTNHHCGYGAIQSQSTVDHDYLRDGFVSRTMGEELPIPGLSVKYLRKIVKVTDKVEGQLKGITDEMERLRKAQEVCQELAKKENADENQLCIVEPFYSNNEYFLIVYDVFKDVRMVFAPPSSVGKFGGDTDNWMWPRHTGDFSVFRVYAGADNRPAEYSKDNKPYKPVYFAAVSMQGYKADDYAMTIGFPGSTDRYLTSWGVEDRIENENNPRIEVRGIKQGIWKEAMSADQATRIKYASKYAQSANYWKNSIGMNRGLARLDVIGRKRAEERAFADWIRKNGKSAVYGDVLSSLEKAYKEGAKANREMTYLSETLFGGTEVVRFAQFANALATNPDAHAGILKSLDDKYKDYLPSLDRKVLPAMLDIVRRRIPADKLPDIFKNVIDKKFKGDTKKYADFVFDKSVVPYSDKFHAMLKSMDKEKFAKAIEKDPAVELSKSVIAAARAIQADAMANAYAIEKGKRLFFAGLREMYPGRALPSDANFTMRMSYGSIKGYEPQDGAWYNYHTTGKGVLEKQDPKSDEFAVQENILDLFRTKNYGRYAENGQLHIAFLSNNDITGGNSGSPVFDKNGRLIGLAFDGNWEAMSGDIEFEPDLQRTISVDIRYVLFMIDKWGQCPRLIQELKLI

SEQ ID NO: 12 - protein, 699 aa, Porphyromonas gingivalis
  Dipeptidyl peptidase 11 (DPP11) (1)..(699): UniProt Accession No. B2RID1
DEGMWLMQQLGRKYAQMKERGLKMKEYDLYNPNGTSLKDAVVLFDGGCTGEVVSDRGLVLTNHHCGYDMIQAHSTLEHNYLENGFWAMREADELPNKDISVVFIDKIEDVTDYVKKELKAIKDPNSMDYLSPKYLQKLADKKAGKNFSAKNPGLSVEIKAFYGGNLYLMFTKKTYTDVRLVGAPPSSIGKFGADTDNWIWPRHTGDFSIFRIYADKNGNPAPYSEDNVPLKPKRFFNISLGGVQENDYAMIMGFPGTTHRYFTASEVDEWKSIDNDIRIRMRDIRQGVMLREMLADPQIKIMYSAKYAASQNAYKRAIGANWAIKTRGLRQNKQAMQDRLIAWGAKQGTPRYEEAVHEIDATVAKRADLRRRYWMIEEGIIRGIEFARSPIPTEDETKALQGNDASARKEAIDKIRTRYSKFANKDYSAEVDKKVAVAMLTEYLKEIPYENLPLHLRLVKDRFAGDVQAYVDDIFARSVFGSEAQFDAFAAVPSVEKLAEDPMVLFASSVFDEYRKLYNELRPYDDPILRAQRTYIAGLLEMDGDQDQFPDANLTLRFTYGQVKGYSPRDNVYYGHQTTLDGVMEKEDPDNWEFVVDPKLKAVYERKDFGRYADRSGRMPVAFCATTHTTGGNSGSPVMNANGELIGLNFDRNWEGVGGDIQYLADYQRSIIVDIRYVLLVIDKVGGCQRLLDEMNIVP

SEQ ID NO: 13 - protein, 698 aa, Pseudoxanthomonas mexicana
  Dipeptidyl Aminopeptidase BII (DAP BII) (1)..(698): UniProt Accession No. V5YM14
GEGMWVPQQLPEIAGPLKKAGLKLSPQQISDLTGDPMGAVVALGGCTASFVSPNGLVVTNHHCAYGAIQLNSTAENNLIKNGFNAPTTADEVSAGPNARVFVLDEITDVTKDAKAAIAAAGDDALARTKALEAFEKKLIADCEAEAGFRCRLYSFSGGNTYRLFKNLEIKDVRLAYAPPGSVGKFGGDIDNWMWPRHTGDFAFYRAYVGKDGKPAAFSKDNVPYQPKHWLKFADQPLGAGDFVMVAGYPGSTNRYALAAEFDNTAQWTYPTIARHYKNQIAMVEAAGKQNADIQVKYAATMAGWNNTSKNYDGQLEGFKRIDAAGQKLREEAAVLGWLKGQGAKGQPALDAHAKLLDLLEQSKATRDRDLTLALFNNTAMLGSATQLYRLSIEREKPNAERESGYQERDLPAIEGGLKQLERRYVAAMDRQLQEYWLNEYIKLPADQRVAAVDAWLGGNDAAAVKRALDRLAGTKLGSTEERLKWFAADRKAFEASNDPAIQYAVAVMPTLLKLEQERKTRAGENLAARPVYLQALADYKKSQGEFVYPDANLSLRITFGNVMGYAPKDGMEYTPFTTLEGVVAKETGQDPFDSPKALLDAVAAKRYGGLEDKRIGSVPVNYLSDLDITGGNSGSPVLDAHGKLVGLAFDGNWESVSSNWVFDPKMTRMIAVDGRYLRWIMQEVYPAPQLLKEMNVGK

SEQ ID NO: 14 - protein, 696 aa, Porphyromonas endodontalis
  Dipeptidyl peptidase 11 (DPP11) (1)..(696): UniProt Accession No. F8WQK8
DGGMWLMQQINGQVARMKSLGMQLEAADIYNPNGSSLKDAVVMFDGGCTGVLVSNQGLLLTNHHCGYDQIQKHSSVQHNYLKDGFWSYSLAEELVNPGLEVEIVDEITDVTAAVKKELERIKKPSGLEFLSPRYLSSLAPEIVGKKAASRPGYRYEIKAFYGGNRYYMFTKKVFRDVRLVAAPPSSIGKFGSDTDNWAWPRHTGDFSIFRLYADKNGNPAEYSKDNVPYRPKRWVKVNAQGVKEGDFALIMGYPGTTYKFFTADEVTEWSEIDNNIRIEMRGILQDVMLREMLADPKINIMYAAKYASSQNGYKRAQGANWAIRRRSLREIKLAQQQEVLAWAKQKGIATTEEAVRAISKAIEGRQDLRMRQRYLLEGILMGIEMSNAPAADSDIADHWDDPARREAGLQSIRKQFEAFFNKDYSPEVEKDQLAIALLTRYAERIPAEKQPISIREGIAEYGSAKAYVEMIFDKSIYASRERFEEFMKNPDRDRLLRDPMSRFAASVAYEHQKLAKEVAAFDAPLAAAQRSYVASVLDMKGQPNLAPDANLTLRFTYGEIKGYQPRDVVTYGAKSTLEGVMEKEDPNNWEYVVDPKLKALYEAKNYGRYANSDGSMPVNFCATTHTTGGNSGSPVMNARGELIGLNFDRNWEGVGGDIEYLPNYQRSIILDIRYLLFIIDKFAGCQRLIDEIQPQF

SEQ ID NO: 15 - protein, 738 aa, Rattus norvegicus
  Dipeptidyl peptidase 3 (DPP3) (1)..(738): UniProt Accession No. O55096
MADTQYILPNDIGVSSLDCREAFRLLSPTERLYAHHLSRAAWYGGLAVLLQTSPEAPYIYALLSRLFRAQDPDQLRQHALAEGLTEEEYQAFLVYAAGVYSNMGNYKSFGDTKFVPNLPKEKLERVILGSKAAQQHPEEVRSLWQTCGELMFSLEPRLRHLGLGKEGVTTYFSGDCAMEDAKLAQDFLDSQNLSAYNTRLFKVVGQEGKYHYEVRLASVLNTEPALDSELTSKLKSYEFQGNHFQVTRGDYAPILQKVVEHLEKAKAYAANSHQEQMLAQYVESFTQGSIEAHKRGSRFWIQDKGPIVESYIGFIESYRDPFGSRGEFEGFVAMVNKDMSAKFERLVASAEQLLKELPWPPAFEKDKFLTPDFTSLDVLTFAGSGIPAGINIPNYDDLRQTEGFKNVSLGNVLAVAYATKREKLTFMEEEDKDLYIRWKGPSFDVQVGLHELLGHGSGKLFVQDEKGAFNFDQETVINPETGEQIQSWYRSGETWDSKFSTIASSYEECRAESVGLYLCLNPQVLQIFGFEGTDAEDVIYVNWLNMVRAGLLALEFYTPETANWRQAHMQARFVILRVLLEAGEGLVTVTPTTGSDGRPDARVHLDRSKIRSVGKPALERFLRRLQVLKSTGDVVAGRALYEGYAAVTDAPPECFLTLRDTVLLRKESRKLIVQPNTRLEGSEVQLVEYEASAAGLIRSFCERFPEDGPELEEVLTQLATADAQFWRDQVQEAPSGQA

SEQ ID NO: 16 - protein, 660 aa, Porphyromonas gingivalis
  Dipeptidyl peptidase 5 (DPP5) (1)..(660): Uniprot accession B2RIT0
TNTGEHLTPELFMTLSRVSEMALSPDGKTAVYAVSFPDVKTNKATRELFTVNLDGSGRKQITDTESNEYAPAWMADGKRIAFMSNEGGSMQLWVMNADGTERRQLSNIEGGITGFLFSPDEKQVLFTKDIKFGKRTKDIYPDLDKATGRIITDLMYKHWDEWVETIPHPFIANATDGMITTGKDIMEGEPYEAPMKPWSGIEDFSWSPDGQNIAYASRKKTGMAYSLSTNSDIYIYNLTSGRTHNISEGMMGYDTYPKFSPDGKSIAWISMERDGYESDLKRLFVADLATGKRTHVNPTFDYNVDMIQWAPDSKGIYFLACKEAETNLWEITLKTGKIRQITQGQHDYADFSVRNDVMLAKRHSFELPDDLYRVNPKNGAAQAVTAENKAILDRLTPIACEKRWMKTTDGGNMLTWVVLPPDFDKNKKYPAILYCQGGPQNTVSQFWSFRWNLRLMAEQGYIVIAPNRHGVPGFGQKWNEQISGDYGGQNMRDYLTAVDEMKKEPYVDGDRIGAVGASYGGFSVYWLAGHHDKRFAAFIAHAGIFNLEMQYATTEEMWFANWDIGGPFWEKDNVVAQRTYATSPHKYVQNWDTPILMIHGELDFRILASQAMAAFDAAQLRGVPSEMLIYPDENHWVLQPQNALLFHRTFFGWLDRWLKK

SEQ ID NO: 17 - protein, 698 aa, Artificial Sequence
  Modified Dipeptidyl Aminopeptidase BII (DAP BII)
GEGMWVPQQLPEIAGPLKKAGLKLSPQQISDLTGDPMGAVVALGGCTASFVSPNGLVVTNHHCAYGAIQLNSTAENNLIKNGFNAPTTADEVSAGPNARVFVLDEITDVTKDAKAAIAAAGDDALARTKALEAFEKKLIADCEAEAGFRCRLYSFSGGNTYRLFKNLEIKDVRLAYAPPGSVGKFGGVASLGMWPSHTGDFAFYRAYVGKDGKPAAFSKDNVPYQPKHWLKFADQPLGAGDFVMVAGYPGSTNRYALAAEFDNTAQWTYPTIARHYKNQIAMVEAAGKQNADIQVKYAATMWGWNNTSKKYDGQLEGFKRIDAAGQKLREEAAVLGWLKGQGAKGQPALDAHAKLLDLLEQSKATRDRDLTLALFNNTAMLGSATQLYRLSIEREKPNAERESGYQERDLPAIEGGLKQLERRYVAAMDRQLQEYWLNEYIKLPADQRVAAVDAWLGGNDAAAVKRALDRLAGTKLGSTEERLKWFAADRKAFEASNDPAIQYAVAVMPTLLKLEQERKTRAGENLAARPVYLQALADYKKSQGEFVYPDANLSLRITFGNVMGYAPKDGMEYTPFTTLEGVVAKETGQDPFDSPKALLDAVAAKRYGGLEDKRIGSVPVNYLSDLDITGGNSGSPVLDAHGKLVGLAFAGNWESVSSNWVFDPKMTRMIAVDGRYLRWIMQEVYPAPQLLKEMNVGK

SEQ ID NO: 18 - protein, 698 aa, Artificial Sequence
  Modified Dipeptidyl Aminopeptidase BII (DAP BII)
GEGMWVPQQLPEIAGPLKKAGLKLSPQQISDLTGDPMGAVVALGGCTASFVSPNGLVVTNHHCAYGAIQLNSTAENNLIKNGFNAPTTADEVSAGPNARVFVLDEITDVTKDAKAAIAAAGDDALARTKALEAFEKKLIADCEAEAGFRCRLYSFSGGNTYRLFKNLEIKDVRLAYAPPGSVGKFGGDIDMGMWPTHTGDFAFYRAYVGKDGKPAAFSKDNVPYQPKHWLKFADQPLGAGDFVMVAGYPGSTNRYALAAEFDNTAQWTYPTIARHYKNQIAMVEAAGKQNADIQVKYAATMAGWNRTSKNYDGQLEGFKRIDAAGQKLREEAAVLGWLKGQGAKGQPALDAHAKLLDLLEQSKATRDRDLTLALFNNTAMLGSATQLYRLSIEREKPNAERESGYQERDLPAIEGGLKQLERRYVAAMDRQLQEYWLNEYIKLPADQRVAAVDAWLGGNDAAAVKRALDRLAGTKLGSTEERLKWFAADRKAFEASNDPAIQYAVAVMPTLLKLEQERKTRAGENLAARPVYLQALADYKKSQGEFVYPDANLSLRITFGNVMGYAPKDGMEYTPFTTLEGVVAKETGQDPFDSPKALLDAVAAKRYGGLEDKRIGSVPVNYLSDLDITGGNSGSPVLDAHGKLVGLAFAGNWESVSSNWVFDPKMTRMIAVDGRYLRWIMQEVYPAPQLLKEMNVGK

SEQ ID NO: 19 - protein, 698 aa, Artificial Sequence
  Modified Dipeptidyl Aminopeptidase BII (DAP BII)
GEGMWVPQQLPEIAGPLKKAGLKLSPQQISDLTGDPMGAVVALGGCTASFVSPNGLVVTNHHCAYGAIQLNSTAENNLIKNGFNAPTTADEVSAGPNARVFVLDEITDVTKDAKAAIAAAGDDALARTKALEAFEKKLIADCEAEAGFRCRLYSFSGGNTYRLFKNLEIKDVRLAYAPPGSVGKFGGDIDMGMWPVHTGDFAFYRAYVGKDGKPAAFSKDNVPYQPKHWLKFADQPLGAGDFVMVAGYPGSTNRYALAAEFDNTAQWTYPTIARHYKNQIAMVEAAGKQNADIQVKYAATMAGWNRTSKNYDGQLEGFKRIDAAGQKLREEAAVLGWLKGQGAKGQPALDAHAKLLDLLEQSKATRDRDLTLALFNNTAMLGSATQLYRLSIEREKPNAERESGYQERDLPAIEGGLKQLERRYVAAMDRQLQEYWLNEYIKLPADQRVAAVDAWLGGNDAAAVKRALDRLAGTKLGSTEERLKWFAADRKAFEASNDPAIQYAVAVMPTLLKLEQERKTRAGENLAARPVYLQALADYKKSQGEFVYPDANLSLRITFGNVMGYAPKDGMEYTPFTTLEGVVAKETGQDPFDSPKALLDAVAAKRYGGLEDKRIGSVPVNYLSDLDITGGNSGSPVLDAHGKLVGLAFAGNWESVSSNWVFDPKMTRMIAVDGRYLRWIMQEVYPAPQLLKEMNVGK

SEQ ID NO: 20 - protein, 722 aa, Pseudoxanthomonas mexicana
  Dipeptidyl Aminopeptidase BII (DAP BII) with Signal Sequence (1)..(722): UniProt Accession No. V5YM14
MRPNLLAAAIAVPLSLLAAQIAQAGEGMWVPQQLPEIAGPLKKAGLKLSPQQISDLTGDPMGAVVALGGCTASFVSPNGLVVTNHHCAYGAIQLNSTAENNLIKNGFNAPTTADEVSAGPNARVFVLDEITDVTKDAKAAIAAAGDDALARTKALEAFEKKLIADCEAEAGFRCRLYSFSGGNTYRLFKNLEIKDVRLAYAPPGSVGKFGGDIDNWMWPRHTGDFAFYRAYVGKDGKPAAFSKDNVPYQPKHWLKFADQPLGAGDFVMVAGYPGSTNRYALAAEFDNTAQWTYPTIARHYKNQIAMVEAAGKQNADIQVKYAATMAGWNNTSKNYDGQLEGFKRIDAAGQKLREEAAVLGWLKGQGAKGQPALDAHAKLLDLLEQSKATRDRDLTLALFNNTAMLGSATQLYRLSIEREKPNAERESGYQERDLPAIEGGLKQLERRYVAAMDRQLQEYWLNEYIKLPADQRVAAVDAWLGGNDAAAVKRALDRLAGTKLGSTEERLKWFAADRKAFEASNDPAIQYAVAVMPTLLKLEQERKTRAGENLAARPVYLQALADYKKSQGEFVYPDANLSLRITFGNVMGYAPKDGMEYTPFTTLEGVVAKETGQDPFDSPKALLDAVAAKRYGGLEDKRIGSVPVNYLSDLDITGGNSGSPVLDAHGKLVGLAFDGNWESVSSNWVFDPKMTRMIAVDGRYLRWIMQEVYPAPQLLKEMNVGK

SEQ ID NO: 21 - protein, 4 aa, Artificial Sequence
  Test peptide
AAAR

SEQ ID NO: 22 - protein, 19 aa, Artificial Sequence
  Test peptide
  MISC_FEATURE (19)..(19): 3' azide
AAGVAMPGAEDDVVGSGSK

SEQ ID NO: 23 - protein, 698 aa, Artificial Sequence
  Modified Dipeptidyl Aminopeptidase BII (DAP BII)
GEGMWVPQQLPEIAGPLKKAGLKLSPQQISDLTGDPMGAVVALGGCTASFVSPNGLVVTNHHCAYGAIQLNSTAENNLIKNGFNAPTTADEVSAGPNARVFVLDEITDVTKDAKAAIAAAGDDALARTKALEAFEKKLIADCEAEAGFRCRLYSFSGGNTYRLFKNLEIKDVRLAYAPPGSVGKFGGDIDMGMWPTHTGDFAFYRAYVGKDGKPAAFSKDNVPYQPKHWLKFADQPLGAGDFVMVAGYPGSTNRYALAAEFDNTAQWTYPTIARHYKNQIAMVEAAGKQNADIQVKYAATMAGWNRKSKNYDGQLEGFKRIDAAGQKLREEAAVLGWLKGQGAKGQPALDAHAKLLDLLEQSKATRDRDLTLALFNNTAMLGSATQLYRLSIEREKPNAERESGYQERDLPAIEGGLKQLERRYVAAMDRQLQEYWLNEYIKLPADQRVAAVDAWLGGNDAAAVKRALDRLAGTKLGSTEERLKWFAADRKAFEASNDPAIQYAVAVMPTLLKLEQERKTRAGENLAARPVYLQALADYKKSQGEFVYPDANLSLRITFGNVMGYAPKDGMEYTPFTTLEGVVAKETGQDPFDSPKALLDAVAAKRYGGLEDKRIGSVPVNYLSDLDITGGNSGSPVLDAHGKLVGLAFAGNWESVSSNWVFDPKMTRMIAVDGRYLRWIMQEVYPAPQLLKEMNVGK

SEQ ID NO: 24 - protein, 698 aa, Artificial Sequence
  Modified Dipeptidyl Aminopeptidase BII (DAP BII)
GEGMWVPQQLPEIAGPLKKAGLKLSPQQISDLTGDPMGAVVALGGCTASFVSPNGLVVTNHHCAYGAIQLNSTAENNLIKNGFNAPTTADEVSAGPNARVFVLDEITDVTKDAKAAIAAAGDDALARTKALEAFEKKLIADCEAEAGFRCRLYSFSGGNTYRLFKNLEIKDVRLAYAPPGSVGKFGGDIDMGMWPTHTGDFAFYRAYVGKDGKPAAFSKDNVPYQPKHWLKFADQPLGAGDFVMVAGYPGSTNRYALAAEFDNTAQWTYPTIARHYKNQIAMVEAAGKQNADIQVKYAATMAGWNRTSKNYDGQLEGFKRIDAAGQKLREEAAVLGWLKGQGAKGQPALDAHAKLLDLLEQSKATRDRDLTLALFNNTAMLGSATQLYRLSIEREKPNAERESGYQERDLPAIEGGLKQLERRYVAAMDRQLQEYWLNEYIKLPADQRVAAVDAWLGGNDAAAVKRALDRLAGTKLGSTEERLKWFAADRKAFEASNDPAIQYAVAVMPTLLKLEQERKTRAGEKLAVRPVYLQALADYKKSQGEFVYPDANLSLRITFGNVMGYAPKDGMEYTPFTTLEGVVAKETGQDPFDSPKALLDAVAVKRYGGLEDKRIGSVPVNYLSDLDITGGNSGSPVLDAHGKLVGLAFAGNWESVSSNWVFDPKMTRMIAVDGRYLRWIMQEVYPAPQLLNEMNVGK

SEQ ID NO: 25 - protein, 698 aa, Artificial Sequence
  Modified Dipeptidyl Aminopeptidase BII (DAP BII)
GEGMWVPQQLPEIAGPLKKAGLKLSPQQISDLTGDPMGAVVALGGCTASFVSPNGLVVTNHHCAYGAIQLNSTAENNLIKNGFNAPTTADEVSAGPNARVFVLDEITDVTKDAKAAIAAAGDDALTRTKALEAFEKKLIADCEAEAGFRCRLYSFSGGNTYRLFKNLEIKDVRLAYAPPGSVGKFGGDIDMGMWPTHTGDFAFYRAYVGKDGKPAAFSKDNVPYQPKHWLKFADQPLVAGDFVMVAGYPGSTNRYALAAEFDNTAQWTYPTIARHYKNQIAMVEAAGKQNADIQVKYAATMAGWNRTSKNYDGQLEGFKRIDAAGQKLREEAAVLGWLKGQGAKGQPALDAHAKLLDLLEQSKATRDRDLTLALFNNTAMLGSATQLYRLSIEREKPNAERESGYQERDLPAIEGGLKQLERRYVAAMDRQLQEYWLNEYIKLPADQRVAAVDAWLGGNDAAAVKRALDRLAGTKLGSTEERLKWFAADRKAFEASNDPAIQYAVAVMPTLLKLEQERKTRAGENLAARPVYLQALADYKKSQGEFVYPDANLSLRITFGNVMGYAPKDGMEYTPFTTLEGVVAKETGQDPFDSPKALLDAVAAKRYGGLEDKRIGSVPVNYLSDLDITGGNSGSPVLDAHGKLVGLAFAGNWESVSSNWVFDPKMTRMIAVDGRYLRWIMQEVYPAPQLLKEMNVGK

SEQ ID NO: 26 - protein, 698 aa, Artificial Sequence
  Modified Dipeptidyl Aminopeptidase BII (DAP BII)
GEGMWVPQQLPEIAGPLKKAGLKLSPQQISDLTGDPMGAVVALGGCTASFVSPNGLVVTNHHCAYGAIQLNSTAENNLIKNGFNAPTTADEVSAGPNARVFVLDEITDVTKDAKAAIAAAGDDALARTKALEAFEKKLIADCEAEAGFRCRLYSFSGGNTYRLFKNLEIKDVRLAYAPPGSVGKFGGDIDMGMWPTHTGDFAFYRAYVGKDGKPAAFSKDNVPYQPKHWLKFADQPLGAGDFVMVAGYPGSTNRYALAAEFDNTAQWTYPTIARHYKNQIAMVEAAGKQNADIQVKYAATMAGWNRTSKNYDGQLEGFKRIDAAGQKLREEAAVLGWLKGQGAKGQPALDAHAKLLDLLEQSKATRDRDLTLALFNNTAMLGSATQLYRLSIEREKPNAERESGYQERDLPAIEGGLKQLERRYVAAMDRQLQEYWLNEYIKLPADQRVAAVDAWLGGNDAAAVKRALDRLAGTKLGSTEERLKWFAADRKAFEASNDPAIQYAVAVMPTLLKLEQERKTRAGENLAARPVYLQALADYKKSQGELVYPDANLSLRITFGNVMGYAPKDGMEYTPFTTLEGVVAKETGQDPFDSPKALLDAVAAKRYGGLEDKRIGSVPVNYLSDLDITGGNSGSPVLDAHGKLVGLAFAGNWESVSSNWVFDPKMTRMIAVDGRYLRWIMQEVYPAPQLLKEMNVGK

SEQ ID NO: 27 - protein, 698 aa, Artificial Sequence
  Modified Dipeptidyl Aminopeptidase BII (DAP BII)
GEGMWVPQQLPEIAGPLKKAGLKLSPQQISDLTGDPMGAVVALGGCTASFVSPNGLVVTNHHCAYGAIQLNSTAENNLIKNGFNAPTTADEVSAGPNARVFVLDEITDVTKDAKAAIAAAGDDALARTKALEAFEKKLIADCEAEAGFRCRLYSFSGGNTYRLFKNLEIKDVRLAYAPPGSVGKFGGDIDMGMWPTHTGDFAFYRAYVGKDGKPAAFSKDNVPYQPKHWLKFADQPLGAGDFVMVAGYPGSTNRYALAAEFDNTAQWTYPTIARHYKNQIAMVEAAGKQNADIQVKYAATMAGWNRTSKNYDGQLEGFKRIDAAGQKLREEAAVLGWLKGQGAKGQPALDAHAKLLDLLEQSKATRDRDLTLALFNNTAMLGSATQLYRLSIEREKPNAERESGYQERDLPAIEGGLKQLERRYVAAMDRQLQEYWLNEYIKLPADQRVAAVDAWLGGNDAAAVKRALDRLAGTKLGSTEERLKWFAADRKAFEASNDPAIQYAVAVMPTLLKLEQERKTRAGENLAARPVYLQALADYKKSQGEFVYPDANLSLRITFGNVMGYAPKDGMEYTPFTTLEGVVAKETGQDPFDSPKALLDAVAAKRYGGLEDKRIGSVPVNYLSDLDITGGNSGSPVLDAHGKLVGLAFAVNWESVSSNWVFDPIMTRMIAVDGRYLRWIMQEVYPAPQLLKEMNVGK

SEQ ID NO: 28 - protein, 698 aa, Artificial Sequence
  Modified Dipeptidyl Aminopeptidase BII (DAP BII)
GEGMWVPQQLPEIAGPLKKAGLKLSPQQISDLTGDPMGAVVALGGCTASFVSPNGLVVTNHHCAYGAIQLNSTAENNLIKNGFNAPTTADEVSAGPNARVFVLDEITDVTKDAKAAIAAAGDDALARTKALEAFEKKLIADCEAEAGFRCRLYSFSGGNTYRLFKNLEIKDVRLAYAPPGSVGKFGGDIDMGMWPTHTGDFAFYRAYVGKDGKPAAFSKDNVPYQPKHWLKFADQPLGAGDFVMVAGYPGSTNRYALAAEFDNTAQWTYPTIARHYKNQIAMVEAAGKQNADIQVKYAATMAGWNRTSKNYDGQLEGFKRIDAAGQKLREEAAVLGWLKGQGAKGQPALDAHAKLLDLLEQSKATRDRDLTLALFNNTAMLGSATQLYRLSIEREKPNAERESGYQERDLPAIEGGLKQLERRYVAAMDRQLQEYWLNEYIKLPADQRVAAVDAWLGGNDAAAVKRALDRLAGTKLGSTEERLKWFAADRKAFEASNDPAIQYAVAVMPTLLKLEQERKTRAGENLAARPVYLQALADYKKSQGEFVYPDANLSLRITFGNVMGYAPKDGMEYTPFTTLEGVVAKETGQDPFDSPKALLDAVAAKRYGGLEDKRIGSVPVNYLSDLDITGGNSGSPVLDAHGKLVGLAFAVNWESVSSNWVFDPKMTRMIAVDGRYLRWIMQEVYPAPQLLKEMNVGK

SEQ ID NO: 29 - protein, 7 aa, Artificial Sequence
  Test Peptide
GRFSGIY

SEQ ID NO: 30 - protein, 7 aa, Artificial Sequence
  Test Peptide
WTQIFGA

SEQ ID NO: 31 - protein, 700 aa, Thermomonas hydrothermalis
  MISC_FEATURE (1)..(700): Dipeptidyl peptidase (Peptidase S46) without the signal peptide
DEGMWVPQQLPEIAGALKKAGLKLDPKQLSDLTGDPMGAVVSLGGCTGSFVSPQGLVATNHHCAYGAIQLNSTPEKNLIKDGFNAPTQADELSAGPNARIYVLEGITDVTAQAKAAMAAAGNDPVARANALEAFEKKITSDCEAEPGYRCRVYSFMGGITYRLFKNLEIKDVRLVYAPPSSVGKFGGDIDNWMWPRHTGDFSFYRAYVGKDGKPAPYSKDNVPYRPKHWLKIADTPLGEGDFVMVAGYPGRTDRYALVAEFENTQNWLYPAISKAYKDQIALVEAAAKDNPEIAVKYAAALAGWNNTSKNFDGQLEGFKRNDVLAIKRREEAAVLEWLRARGKAGTPALEAHAALVKLVADTARTQERDLVLGSFNRTGIIGVAVNLYRLAIERQKPDAEREPGYQQRDLPVIEGSLKQMERRYVPAMDRQLRAYWLDRYVALPAAQHVAAVDAWLGGSDKAAAEAALARLDQSRLGSLEERLKWFNADRAAFEASTDPAIQYAVAVMPTLLAMEQQAKTRYGVALEARPRYLQAVVDYKKSKGQAVYPDANSTLRITYGHVKGYTGLNGKVYTPFTTLEEVAAKETGVEPFDNPKALLEAVAAKRYAGLADARLGTVPVNFLADLDITGGNSGSPVLDANGRLVGLAFDGTLESVASNWVFDPVLTRMISVDQRYMRWIMQEVMPAPQLLEELGVPPRQ

SEQ ID NO: 32 - protein, 692 aa, Caldithrix abyssi
  MISC_FEATURE (1)..(692): Dipeptidyl peptidase (S46 family peptidase) without the signal peptide
EEGMYPITEIHKLNLKKLGIELSADQIFSENEVSLSDAIVQIGGCTGSFISPEGLILTNHHCAFRAIQNISSTENDYLTNGFVAHTLQEERPAKGYTVRITERVEDVSQRVLNAVKHIEDPIEREKAIEKITKQIVKEQEQKHPGKRAAVSEMFPGKTYYLFIYTYLKDVRLVYAPPRSIGEFGGEFDNWEWPRHTGDFTLMRAYVAPDGSPSDYSEENVPYRPKSYLKVAAKGVEEGDRVFILGYPGRTYRHRTSAFLAFEYEFRMPFVVDWYQWQIDLLTTLGKDDADRSLKFSSWIKGLANTEKNYRGKLQGIRRIGLLEQKKNEEEKIQVFIAENNLKKYQHVLTEIKQIYHTYRQSAVREMLLSYFGRSPVLPAVARTLVLAAEERQKEDLERERAFMDRNFKRTQTYTLLRLKNFDSQADQLILQELLKKAAALPEDQRISALRSIFKLDDAAETRQVISEAYRKTRLSDPEFVKTCFAKTPDELKALNDPLINWMLALKEDYETLKNIRKERNGKLRRLRALWLEAKQAYLKTDFIPDANGTYRMTFGFIEGYAPADAVYKAPITTGRGILEKHTGKSPFDTPEKLLALLKAKQFGPFVSKTVGTLPVGILYSCDTTGGNSGSPVLNARGQLVGLNFDRAFEATINDYAWNHQYSRSIGVDIRYILFLLKYFSGAEHLLEEMGVQ

SEQ ID NO: 33 - protein, 723 aa, Thermomonas hydrothermalis
  MISC_FEATURE (1)..(723): Dipeptidyl peptidase (Peptidase S46) with the signal peptide
MHKTRLVAALAAALATLAPAAWADEGMWVPQQLPEIAGALKKAGLKLDPKQLSDLTGDPMGAVVSLGGCTGSFVSPQGLVATNHHCAYGAIQLNSTPEKNLIKDGFNAPTQADELSAGPNARIYVLEGITDVTAQAKAAMAAAGNDPVARANALEAFEKKITSDCEAEPGYRCRVYSFMGGITYRLFKNLEIKDVRLVYAPPSSVGKFGGDIDNWMWPRHTGDFSFYRAYVGKDGKPAPYSKDNVPYRPKHWLKIADTPLGEGDFVMVAGYPGRTDRYALVAEFENTQNWLYPAISKAYKDQIALVEAAAKDNPEIAVKYAAALAGWNNTSKNFDGQLEGFKRNDVLAIKRREEAAVLEWLRARGKAGTPALEAHAALVKLVADTARTQERDLVLGSFNRTGIIGVAVNLYRLAIERQKPDAEREPGYQQRDLPVIEGSLKQMERRYVPAMDRQLRAYWLDRYVALPAAQHVAAVDAWLGGSDKAAAEAALARLDQSRLGSLEERLKWFNADRAAFEASTDPAIQYAVAVMPTLLAMEQQAKTRYGVALEARPRYLQAVVDYKKSKGQAVYPDANSTLRITYGHVKGYTGLNGKVYTPFTTLEEVAAKETGVEPFDNPKALLEAVAAKRYAGLADARLGTVPVNFLADLDITGGNSGSPVLDANGRLVGLAFDGTLESVASNWVFDPVLTRMISVDQRYMRWIMQEVMPAPQLLEELGVPPRQ

SEQ ID NO: 34 - protein, 710 aa, Caldithrix abyssi
  MISC_FEATURE (1)..(710): Dipeptidyl peptidase  (S46 family peptidase) with the signal peptide
MKIRLFGVLLLFTFSLFAEEGMYPITEIHKLNLKKLGIELSADQIFSENEVSLSDAIVQIGGCTGSFISPEGLILTNHHCAFRAIQNISSTENDYLTNGFVAHTLQEERPAKGYTVRITERVEDVSQRVLNAVKHIEDPIEREKAIEKITKQIVKEQEQKHPGKRAAVSEMFPGKTYYLFIYTYLKDVRLVYAPPRSIGEFGGEFDNWEWPRHTGDFTLMRAYVAPDGSPSDYSEENVPYRPKSYLKVAAKGVEEGDRVFILGYPGRTYRHRTSAFLAFEYEFRMPFVVDWYQWQIDLLTTLGKDDADRSLKFSSWIKGLANTEKNYRGKLQGIRRIGLLEQKKNEEEKIQVFIAENNLKKYQHVLTEIKQIYHTYRQSAVREMLLSYFGRSPVLPAVARTLVLAAEERQKEDLERERAFMDRNFKRTQTYTLLRLKNFDSQADQLILQELLKKAAALPEDQRISALRSIFKLDDAAETRQVISEAYRKTRLSDPEFVKTCFAKTPDELKALNDPLINWMLALKEDYETLKNIRKERNGKLRRLRALWLEAKQAYLKTDFIPDANGTYRMTFGFIEGYAPADAVYKAPITTGRGILEKHTGKSPFDTPEKLLALLKAKQFGPFVSKTVGTLPVGILYSCDTTGGNSGSPVLNARGQLVGLNFDRAFEATINDYAWNHQYSRSIGVDIRYILFLLKYFSGAEHLLEEMGVQ

SEQ ID NO: 35 - protein, 190 aa, Mus musculus
  MISC_FEATURE (1)..(190): Lipocalin S066  (Neutrophil Gelatinase-associated Lipocalin)
QDSTQNLIPAPSLLTVPLQPDFRSDQFRGRWYVVGLAGNAVQKKTEGSFTMYSTIYELQENNSYNVTSILVRDQDQGCRYWIRTFVPSSRAGQFTLGNMHRYPQVQSYNVQVATTDYNQFAMVFFRKTSENKQYFKITLYGRTKELSPELKERFTRFAKSLGLKDDNIIFSVPTDQCIDNSAWSHPQFEK

SEQ ID NO: 36 - protein, 698 aa, Artificial Sequence
  Modified Dipeptidyl Aminopeptidase BII (DAP BII)
GEGMWVPQQLPEIAGPLKKAGLKLSPQQISDLTGDPMGAVVALGGCTASFVSPNGLVVTNHHCAYGAIQLNSTAENNLIKNGFNAPTTADEVSAGPNARVFVLDEITDVTKDAKAAIAAAGDDALARTKALEAFEKKLIADCEAEAGFRCRLYSFSGGNTYRLFKNLEIKDVRLAYAPPGSVGKFGGDIDCLMWPKHTGDFAFYRAYVGKDGKPAAFSKDNVPYQPKHWLKFADQPLGAGDFVMVAGYPGSTNRYALAAEFDNTAQWTYPTIARHYKNQIAMVEAAGKQNADIQVKYAATMAGWNRTSKDYDGQLEGFKRIDAAGQKLREEAAVLGWLKGQGAKGQPALDAHAKLLDLLEQSKATRDRDLTLALFNNTAMLGSATQLYRLSIEREKPNAERESGYQERDLPAIEGGLKQLERRYVAAMDRQLQEYWLNEYIKLPADQRVAAVDAWLGGNDAAAVKRALDRLAGTKLGSTEERLKWFAADRKAFEASNDPAIQYAVAVMPTLLKLEQERKTRAGENLAARPVYLQALADYKKSQGEFVYPDANLSLRITFGNVMGYAPKDGMEYTPFTTLEGVVAKETGQDPFDSPKALLDAVAAKRYGGLEDKRIGSVPVNYLSDLDITGGNSGSPVLDAHGKLVGLAFDYNWEGGSSNWVFDPKMTRMIAVDGRYLRWIMQEVYPAPQLLKEMNVGK

SEQ ID NO: 37 - protein, 698 aa, Artificial Sequence
  Modified Dipeptidyl Aminopeptidase BII (DAP BII)
GEGMWVPQQLPEIAGPLKKAGLKLSPQQISDLTGDPMGAVVALGGCTASFVSPNGLVVTNHHCAYGAIQLNSTAENNLIKNGFNAPTTADEVSAGPNARVFVLDEITDVTKDAKAAIAAAGDDALARTKALEAFEKKLIADCEAEAGFRCRLYSFSGGNTYRLFKNLEIKDVRLAYAPPGSVGKFGGDIDCLMWPRHTGDFAFYRAYVGKDGKPAAFSKDNVPYQPKHWLKFADQPLGAGDFVMVAGYPGSTNRYALAAEFDNTAQWTYPTIARHYKNQIAMVEAAGKQNADIQVKYAATMAGWNRTSKDYDGQLEGFKRIDAAGQKLREEAAVLGWLKGQGAKGQPALDAHAKLLDLLEQSKATRDRDLTLALFNNTAMLGSATQLYRLSIEREKPNAERESGYQERDLPAIEGGLKQLERRYVAAMDRQLQEYWLNEYIKLPADQRVAAVDAWLGGNDAAAVKRALDRLAGTKLGSTEERLKWFAADRKAFEASNDPAIQYAVAVMPTLLKLEQERKTRAGENLAARPVYLQALADYKKSQGEFVYPDANLSLRITFGNVMGYAPKDGMEYTPFTTLEGVVAKETGQDPFDSPKALLDAVAAKRYGGLEDKRIGSVPVNYLSDLDITGGNSGSPVLDAHGKLVGLAFDYNWEGGSSNWVFDPKMTRMIAVDGRYLRWIMQEVYPAPQLLKEMNVGK

SEQ ID NO: 38 - protein, 698 aa, Artificial Sequence
  Modified Dipeptidyl Aminopeptidase BII (DAP BII)
GEGMWVPQQLPEIAGPLKKAGLKLSPQQISDLTGDPMGAVVALGGCTASFVSPNGLVVTNHHCAYGAIQLNSTAENNLIKNGFNAPTTADEVSAGPNARVFVLDEITDVTKDAKAAIAAAGDDALARTKALEAFEKKLIADCEAEAGFRCRLYSFSGGNTYRLFKNLEIKDVRLAYAPPGSVGKFGGDIDFFMWPRHTGDFAFYRAYVGKDGKPAAFSKDNVPYQPKHWLKFADQPLGAGDFVMVAGYPGSTNRYALAAEFDNTAQWTYPTIARHYKNQIAMVEAAGKQNADIQVKYAATMAGWNRTSKGYDGQLEGFKRIDAAGQKLREEAAVLGWLKGQGAKGQPALDAHAKLLDLLEQSKATRDRDLTLALFNNTAMLGSATQLYRLSIEREKPNAERESGYQERDLPAIEGGLKQLERRYVAAMDRQLQEYWLNEYIKLPADQRVAAVDAWLGGNDAAAVKRALDRLAGTKLGSTEERLKWFAADRKAFEASNDPAIQYAVAVMPTLLKLEQERKTRAGENLAARPVYLQALADYKKSQGEFVYPDANLSLRITFGNVMGYAPKDGMEYTPFTTLEGVVAKETGQDPFDSPKALLDAVAAKRYGGLEDKRIGSVPVNYLSDLDITGGNSGSPVLDAHGKLVGLAFDHNWESESSNWVFDPKMTRMIAVDGRYLRWIMQEVYPAPQLLKEMNVGK

SEQ ID NO: 39 - protein, 698 aa, Artificial Sequence
  Modified Dipeptidyl Aminopeptidase BII (DAP BII)
GEGMWVPQQLPEIAGPLKKAGLKLSPQQISDLTGDPMGAVVALGGCTASFVSPNGLVVTNHHCAYGAIQLNSTAENNLIKNGFNAPTTADEVSAGPNARVFVLDEITDVTKDAKAAIAAAGDDALARTKALEAFEKKLIADCEAEAGFRCRLYSFSGGNTYRLFKNLEIKDVRLAYAPPGSVGKFGGDIDRLMWPRHTGDFAFYRAYVGKDGKPAAFSKDNVPYQPKHWLKFADQPLGAGDFVMVAGYPGSTNRYALAAEFDNTAQWTYPTIARHYKNQIAMVEAAGKQNADIQVKYAATMAGWNSTSKLYDGQLEGFKRIDAAGQKLREEAAVLGWLKGQGAKGQPALDAHAKLLDLLEQSKATRDRDLTLALFNNTAMLGSATQLYRLSIEREKPNAERESGYQERDLPAIEGGLKQLERRYVAAMDRQLQEYWLNEYIKLPADQRVAAVDAWLGGNDAAAVKRALDRLAGTKLGSTEERLKWFAADRKAFEASNDPAIQYAVAVMPTLLKLEQERKTRAGENLAARPVYLQALADYKKSQGEFVYPDANLSLRITFGNVMGYAPKDGMEYTPFTTLEGVVAKETGQDPFDSPKALLDAVAAKRYGGLEDKRIGSVPVNYLSDLDITGGNSGSPVLDAHGKLVGLAFDTNWETSSSNWVFDPKMTRMIAVDGRYLRWIMQEVYPAPQLLKEMNVGK

SEQ ID NO: 40 - protein, 698 aa, Artificial Sequence
  Modified Dipeptidyl Aminopeptidase BII (DAP BII)
GEGMWVPQQLPEIAGPLKKAGLKLSPQQISDLTGDPMGAVVALGGCTASFVSPNGLVVTNHHCAYGAIQLNSTAENNLIKNGFNAPTTADEVSAGPNARVFVLDEITDVTKDAKAAIAAAGDDALARTKALEAFEKKLIADCEAEAGFRCRLYSFSGGNTYRLFKNLEIKDVRLAYAPPGSVGKFGGDIDSWMWPHHTGDFAFYRAYVGKDGKPAAFSKDNVPYQPKHWLKFADQPLGAGDFVMVAGYPGSTNRYALAAEFDNTAQWTYPTIARHYKNQIAMVEAAGKQNADIQVKYAATMAGWNATSKNYDGQLEGFKRIDAAGQKLREEAAVLGWLKGQGAKGQPALDAHAKLLDLLEQSKATRDRDLTLALFNNTAMLGSATQLYRLSIEREKPNAERESGYQERDLPAIEGGLKQLERRYVAAMDRQLQEYWLNEYIKLPADQRVAAVDAWLGGNDAAAVKRALDRLAGTKLGSTEERLKWFAADRKAFEASNDPAIQYAVAVMPTLLKLEQERKTRAGENLAARPVYLQALADYKKSQGEFVYPDANLSLRITFGNVMGYAPKDGMEYTPFTTLEGVVAKETGQDPFDSPKALLDAVAAKRYGGLEDKRIGSVPVNYLSDLDITGGNSGSPVLDAHGKLVGLAFGGNWESVSSNWVFDPKMTRMIAVDGRYLRWIMQEVYPAPQLLKEMNVGK

SEQ ID NO: 41 - protein, 698 aa, Artificial Sequence
  Modified Dipeptidyl Aminopeptidase BII (DAP BII)
GEGMWVPQQLPEIAGPLKKAGLKLSPQQISDLTGDPMGAVVALGGCTASFVSPNGLVVTNHHCAYGAIQLNSTAENNLIKNGFNAPTTADEVSAGPNARVFVLDEITDVTKDAKAAIAAAGDDALARTKALEAFEKKLIADCEAEAGFRCRLYSFSGGNTYRLFKNLEIKDVRLAYAPPGSVGKFGGDIDTWMWPHHTGDFAFYRAYVGKDGKPAAFSKDNVPYQPKHWLKFADQPLGAGDFVMVAGYPGSTNRYALAAEFDNTAQWTYPTIARHYKNQIAMVEAAGKQNADIQVKYAATMAGWNATSKNYDGQLEGFKRIDAAGQKLREEAAVLGWLKGQGAKGQPALDAHAKLLDLLEQSKATRDRDLTLALFNNTAMLGSATQLYRLSIEREKPNAERESGYQERDLPAIEGGLKQLERRYVAAMDRQLQEYWLNEYIKLPADQRVAAVDAWLGGNDAAAVKRALDRLAGTKLGSTEERLKWFAADRKAFEASNDPAIQYAVAVMPTLLKLEQERKTRAGENLAARPVYLQALADYKKSQGEFVYPDANLSLRITFGNVMGYAPKDGMEYTPFTTLEGVVAKETGQDPFDSPKALLDAVAAKRYGGLEDKRIGSVPVNYLSDLDITGGNSGSPVLDAHGKLVGLAFGGNWESVSSNWVFDPKMTRMIAVDGRYLRWIMQEVYPAPQLLKEMNVGK

SEQ ID NO: 42 - protein, 698 aa, Artificial Sequence
  Modified Dipeptidyl Aminopeptidase BII (DAP BII)
GEGMWVPQQLPEIAGPLKKAGLKLSPQQISDLTGDPMGAVVALGGCTASFVSPNGLVVTNHHCAYGAIQLNSTAENNLIKNGFNAPTTADEVSAGPNARVFVLDEITDVTKDAKAAIAAAGDDALARTKALEAFEKKLIADCEAEAGFRCRLYSFSGGNTYRLFKNLEIKDVRLAYAPPGSVGKFGGDIDMWMWPHHTGDFAFYRAYVGKDGKPAAFSKDNVPYQPKHWLKFADQPLGAGDFVMVAGYPGSTNRYALAAEFDNTAQWTYPTIARHYKNQIAMVEAAGKQNADIQVKYAATMAGWNATSKNYDGQLEGFKRIDAAGQKLREEAAVLGWLKGQGAKGQPALDAHAKLLDLLEQSKATRDRDLTLALFNNTAMLGSATQLYRLSIEREKPNAERESGYQERDLPAIEGGLKQLERRYVAAMDRQLQEYWLNEYIKLPADQRVAAVDAWLGGNDAAAVKRALDRLAGTKLGSTEERLKWFAADRKAFEASNDPAIQYAVAVMPTLLKLEQERKTRAGENLAARPVYLQALADYKKSQGEFVYPDANLSLRITFGNVMGYAPKDGMEYTPFTTLEGVVAKETGQDPFDSPKALLDAVAAKRYGGLEDKRIGSVPVNYLSDLDITGGNSGSPVLDAHGKLVGLAFGGNWESVSSNWVFDPKMTRMIAVDGRYLRWIMQEVYPAPQLLKEMNVGK

SEQ ID NO: 43 - protein, 698 aa, Artificial Sequence
  Modified Dipeptidyl Aminopeptidase BII (DAP BII)
GEGMWVPQQLPEIAGPLKKAGLKLSPQQISDLTGDPMGAVVALGGCTASFVSPNGLVVTNHHCAYGAIQLNSTAENNLIKNGFNAPTTADEVSAGPNARVFVLDEITDVTKDAKAAIAAAGDDALARTKALEAFEKKLIADCEAEAGFRCRLYSFSGGNTYRLFKNLEIKDVRLAYAPPGSVGKFGGDIDVWMWPRHTGDFAFYRAYVGKDGKPAAFSKDNVPYQPKHWLKFADQPLGAGDFVMVAGYPGSTNRYALAAEFDNTAQWTYPTIARHYKNQIAMVEAAGKQNADIQVKYAATMAGWNATSKNYDGQLEGFKRIDAAGQKLREEAAVLGWLKGQGAKGQPALDAHAKLLDLLEQSKATRDRDLTLALFNNTAMLGSATQLYRLSIEREKPNAERESGYQERDLPAIEGGLKQLERRYVAAMDRQLQEYWLNEYIKLPADQRVAAVDAWLGGNDAAAVKRALDRLAGTKLGSTEERLKWFAADRKAFEASNDPAIQYAVAVMPTLLKLEQERKTRAGENLAARPVYLQALADYKKSQGEFVYPDANLSLRITFGNVMGYAPKDGMEYTPFTTLEGVVAKETGQDPFDSPKALLDAVAAKRYGGLEDKRIGSVPVNYLSDLDITGGNSGSPVLDAHGKLVGLAFSGNWESVSSNWVFDPKMTRMIAVDGRYLRWIMQEVYPAPQLLKEMNVGK

SEQ ID NO: 44 - protein, 698 aa, Artificial Sequence
  Modified Dipeptidyl Aminopeptidase BII (DAP BII)
GEGMWVPQQLPEIAGPLKKAGLKLSPQQISDLTGDPMGAVVALGGCTASFVSPNGLVVTNHHCAYGAIQLNSTAENNLIKNGFNAPTTADEVSAGPNARVFVLDEITDVTKDAKAAIAAAGDDALARTKALEAFEKKLIADCEAEAGFRCRLYSFSGGNTYRLFKNLEIKDVRLAYAPPGSVGKFGGDIDSWMWPRHTGDFAFYRAYVGKDGKPAAFSKDNVPYQPKHWLKFADQPLGAGDFVMVAGYPGSTNRYALAAEFDNTAQWTYPTIARHYKNQIAMVEAAGKQNADIQVKYAATMAGWNGTSKNYDGQLEGFKRIDAAGQKLREEAAVLGWLKGQGAKGQPALDAHAKLLDLLEQSKATRDRDLTLALFNNTAMLGSATQLYRLSIEREKPNAERESGYQERDLPAIEGGLKQLERRYVAAMDRQLQEYWLNEYIKLPADQRVAAVDAWLGGNDAAAVKRALDRLAGTKLGSTEERLKWFAADRKAFEASNDPAIQYAVAVMPTLLKLEQERKTRAGENLAARPVYLQALADYKKSQGEFVYPDANLSLRITFGNVMGYAPKDGMEYTPFTTLEGVVAKETGQDPFDSPKALLDAVAAKRYGGLEDKRIGSVPVNYLSDLDITGGNSGSPVLDAHGKLVGLAFSGNWESVSSNWVFDPKMTRMIAVDGRYLRWIMQEVYPAPQLLKEMNVGK

SEQ ID NO: 45 - protein, 7 aa, Artificial Sequence
  test peptide
IHAGYAW

SEQ ID NO: 46 - protein, 13 aa, Artificial Sequence
  test peptide
  MISC_FEATURE (1)..(1): Xaa can be any naturally occurring amino acid
XGAEIAGDVAGGK

SEQ ID NO: 47 - protein, 20 aa, Artificial Sequence
  test peptide
LMSHNARGAEDDVVRGGGGK

SEQ ID NO: 48 - protein, 4 aa, Artificial Sequence
  test peptide
LAAR

SEQ ID NO: 49 - protein, 13 aa, Artificial Sequence
  test peptide
AAAEIRGDVRGGK

SEQ ID NO: 50 - protein, 12 aa, Artificial Sequence
  test peptide
AAEIRGDVRGGK

SEQ ID NO: 51 - protein, 5 aa, Artificial Sequence
  test peptide
AAEIR

SEQ ID NO: 52 - protein, 4 aa, Artificial Sequence
  test peptide
GDVR

SEQ ID NO: 53 - protein, 17 aa, Artificial Sequence
  test peptide
  MISC_FEATURE (17)..(17): C-terminal azide modification
GVAMPGAEDDVVGSGSK

SEQ ID NO: 54 - protein, 18 aa, Artificial Sequence
  test peptide
  MISC_FEATURE (18)..(18): C-terminal azide modification
AGVAMPGAEDDVVGSGSK

SEQ ID NO: 55 - protein, 8 aa, Artificial Sequence
  test peptide
LIHAGYAW